European Patent Application EP 4 350 008 A1, published April 10, 2024. Title: Biomarker Combination for Colorectal Cancer Early Diagnosis and Use Thereof. Applicant: Wedo (Suzhou) Biotechnological Co.,Ltd. The sequence listing filed with the application follows.

SEQUENCE LISTING (10 sequences)

SEQ ID NO: 1 - DNA, 21 bp, Artificial Sequence
  Sense primer of primer pair (1)
aagtgttagcggtataggatg

SEQ ID NO: 2 - DNA, 19 bp, Artificial Sequence
  Anti-sense primer of primer pair (1)
cgtgtctcagttccaatgt

SEQ ID NO: 3 - DNA, 20 bp, Artificial Sequence
  Sense primer of primer pair (2)
ggatttattgggcgtaaagc

SEQ ID NO: 4 - DNA, 24 bp, Artificial Sequence
  Anti-sense primer of primer pair (2)
ggcattcctacaaatatctacgaa

SEQ ID NO: 5 - DNA, 22 bp, Artificial Sequence
  Sense primer of primer pair (3)
gcgtagatattaggaggaatac

SEQ ID NO: 6 - DNA, 19 bp, Artificial Sequence
  Anti-sense primer of primer pair (3)
gcggaatgcttaatgtgtt

SEQ ID NO: 7 - DNA, 18 bp, Artificial Sequence
  Sense primer of primer pair (4)
catcgcttaacggtggat

SEQ ID NO: 8 - DNA, 18 bp, Artificial Sequence
  Anti-sense primer of primer pair (4)
ttcgccattggtgttctt

SEQ ID NO: 9 - DNA, 22 bp, Artificial Sequence
  Sense primer of primer pair (5)
gcaggcctaacacatgcaagtc

SEQ ID NO: 10 - DNA, 20 bp, Artificial Sequence
  Anti-sense primer of primer pair (5)
ctgctgcctcccgtaggagt